European Patent Application EP 4 180 515 A1, published May 17, 2023. Title: METHOD FOR INDUCING DIFFERENTIATION OF PLURIPOTENT STEM CELLS INTO MESODERMAL CELLS. Applicant: TOSOH CORPORATION. The sequence listing filed with the application follows.

SEQUENCE LISTING (4 sequences)

SEQ ID NO: 1 - DNA, 36 bp, Homo sapiens
aacgccgagttgagcaaggccggtacttgtagttgg

SEQ ID NO: 2 - DNA, 40 bp, Homo sapiens
aactctccaacatcctgaaccccttctgcgtcacaccatt

SEQ ID NO: 3 - DNA, 41 bp, Homo sapiens
acatcgctcagacaccatgtgtagttgaggtcaatgaaggg

SEQ ID NO: 4 - DNA, 44 bp, Homo sapiens
cgtctccttcagcaaagtcaactatgtggattcgaggctcatac